European Patent Application EP 4 137 520 A1, published February 22, 2023. Title: Anti-HER2 affibody and switchable chimeric antigen receptor using the same as switch molecule. Applicant: AbClon Inc. The sequence listing filed with the application follows.

SEQUENCE LISTING (23 sequences)

SEQ ID NO: 1 - protein, 58 aa, Artificial Sequence
  ZQAA1
VDNKFNKELRVAYWEIVKLPNLNPYQSRAFIRSLYDDPSQSANLLAEAKKLNDAQAPK

SEQ ID NO: 2 - protein, 58 aa, Artificial Sequence
  ZQAA7
VDNKFNKELRGAYWEITSLPNLNHSQITAFIVSLYDDPSQSANLLAEAKKLNDAQAPK

SEQ ID NO: 3 - protein, 58 aa, Artificial Sequence
  ZQAA8
VDNKFNKEMRDAYWEIVRLPNLNPPQSTAFIRSLYDDPSQSANLLAEAKKLNDAQAPK

SEQ ID NO: 4 - protein, 58 aa, Artificial Sequence
  ZQAA11
VDNKFNKEYMLAYWEIVKLPNLNYPQQHAFIRSLFDDPSQSANLLAEAKKLNDAQAPK

SEQ ID NO: 5 - protein, 58 aa, Artificial Sequence
  ZQAA22
VDNKFNKEINKAYWEIISLPNLNKEQHHAFIHSLYDDPSQSANLLAEAKKLNDAQAPK

SEQ ID NO: 6 - protein, 58 aa, Artificial Sequence
  ZQAA1234
VDNKFNKELRVAYWEIVKLPNLNPPQITAFIRSLYDDPSQSANLLAEAKKLNDAQAPK

SEQ ID NO: 7 - protein, 58 aa, Artificial Sequence
  ZQAA1239
VDNKFNKELRVAYWEIVKLPNLNPKQITAFIKQLYDDPSQSANLLAEAKKLNDAQAPK

SEQ ID NO: 8 - protein, 58 aa, Artificial Sequence
  ZQAA8293
VDNKFNKEMRDAYWEIVRLPNLNRIQSVAFIRQLYDDPSQSANLLAEAKKLNDAQAPK

SEQ ID NO: 9 - protein, 5 aa, Artificial Sequence
  CDRH1 of Anti-cotinine antibody
RDWMN

SEQ ID NO: 10 - protein, 15 aa, Artificial Sequence
  CDRH2 of Anti-cotinine antibody
AIGRSGDTYYATWAK

SEQ ID NO: 11 - protein, 11 aa, Artificial Sequence
  CDRH3 of Anti-cotinine antibody
IPYFGWNNGDI

SEQ ID NO: 12 - protein, 13 aa, Artificial Sequence
  CDRL1 of Anti-cotinine antibody
QSSQSPYSNEWLS

SEQ ID NO: 13 - protein, 7 aa, Artificial Sequence
  CDRL2 of Anti-cotinine antibody
RISTLAS

SEQ ID NO: 14 - protein, 12 aa, Artificial Sequence
  CDRL3 of Anti-cotinine antibody
AGGYNFGLFLFG

SEQ ID NO: 15 - protein, 119 aa, Artificial Sequence
  Heavy chain of Anti-cotinine antibody
EVQLVESGGGLVQPGGSLRLSCAASGHLRRRDWMNWVRQAPGKGLEWVAAIGRSGDTYYATWAKGRFTISADTSKNTAYLQMNSLRAEDTAVYYCSRIPYFGWNNGDIWGQGTLVTVSS

SEQ ID NO: 16 - DNA, 357 bp, Artificial Sequence
  Heavy chain of Anti-cotinine antibody
gaggtgcagctggtggagtctggcggcggactggtgcagcctggcggaagcttgcggctgtcctgcgccgcctccgggcatcttcggaggagggactggatgaactgggtgcggcaggcccctggcaagggcctagagtgggtggccgccattggtagaagtggagacacatactacgcgacctgggcgaaaggccggttcaccatctccgccgacacctccaagaacaccgcctacctgcagatgaactccctgcgggccgaggacaccgccgtgtactactgctccagaattccttattttggttggaataatggtgacatctggggccagggcacactcgtgaccgtgtcctcc

SEQ ID NO: 17 - protein, 110 aa, Artificial Sequence
  Light chain of Anti-cotinine antibody
DIQMTQSPSSLSASVGDRVTITCQSSQSPYSNEWLSWYQQKPGKAPKLLIYRISTLASGVPSRFSGSRSGTDFTLTISSLQPEDFATYYCAGGYNFGLFLFGQGTKVEIK

SEQ ID NO: 18 - DNA, 330 bp, Artificial Sequence
  Light chain of Anti-cotinine antibody
gacatccagatgacccagtccccctcctcgctgagcgcctccgtgggcgaccgggtgaccatcacctgccagtccagtcagagtccttatagtaacgagtggttatcctggtatcagcagaagcctggcaaggcgcctaagctgctgatctacaggatatccactctggcatctggcgtgccttcccggttctccggatcccggtccggcaccgacttcaccctgaccatctcctccctgcaacctgaggacttcgccacctactactgcgcaggcggttataattttggtttgtttctcttcggccagggtaccaaggtggagatcaag

SEQ ID NO: 19 - DNA, 1184 bp, Artificial Sequence
  EF-1alpha promoter
tgtgaggctccggtgcccgtcagtgggcagagcgcacatcgcccacagtccccgagaagttggggggaggggtcggcaattgaaccggtgcctagagaaggtggcgcggggtaaactgggaaagtgatgtcgtgtactggctccgcctttttcccgagggtgggggagaaccgtatataagtgcagtagtcgccgtgaacgttctttttcgcaacgggtttgccgccagaacacaggtaagtgccgtgtgtggttcccgcgggcctggcctctttacgggttatggcccttgcgtgccttgaattacttccacctggctgcagtacgtgattcttgatcccgagcttcgggttggaagtgggtgggagagttcgaggccttgcgcttaaggagccccttcgcctcgtgcttgagttgaggcctggcctgggcgctggggccgccgcgtgcgaatctggtggcaccttcgcgcctgtctcgctgctttcgataagtctctagccatttaaaatttttgatgacctgctgcgacgctttttttctggcaagatagtcttgtaaatgcgggccaagatctgcacactggtatttcggtttttggggccgcgggcggcgacggggcccgtgcgtcccagcgcacatgttcggcgaggcggggcctgcgagcgcggccaccgagaatcggacgggggtagtctcaagctggccggcctgctctggtgcctggcctcgcgccgccgtgtatcgccccgccctgggcggcaaggctggcccggtcggcaccagttgcgtgagcggaaagatggccgcttcccggccctgctgcagggagctcaaaatggaggacgcggcgctcgggagagcgggcgggtgagtcacccacacaaaggaaaagggcctttccgtcctcagccgtcgcttcatgtgactccacggagtaccgggcgccgtccaggcacctcgattagttctcgagcttttggagtacgtcgtctttaggttggggggaggggttttatgcgatggagtttccccacactgagtgggtggagactgaagttaggccagcttggcacttgatgtaattctccttggaatttgccctttttgagtttggatcttggttcattctcaagcctcagacagtggttcaaagtttttttcttccatttcaggtgtcgtga

SEQ ID NO: 20 - DNA, 63 bp, Artificial Sequence
  CD8 leader
atggccctgcctgtgaccgctctgctgctgcccctggctctgctgctgcacgccgctcgcccc

SEQ ID NO: 21 - DNA, 207 bp, Artificial Sequence
  CD8 hinge and TM region
accacaactccagctccccggccccctacccctgcaccaacaatcgccagccagcctctgtccctgagaccagaggcatgtaggccagctgcaggaggagcagtgcatacaagaggcctggacttcgcctgcgatatctacatttgggctcctctggcaggaacttgtggcgtgctgctgctgtctctggtcatcaccctgtactgc

SEQ ID NO: 22 - DNA, 126 bp, Artificial Sequence
  CD137
aaaaggggccgcaagaaactgctgtatattttcaagcagcccttcatgcggcccgtgcagaccacacaggaggaagacgggtgctcctgtagattccccgaggaagaggaaggcgggtgtgagctg

SEQ ID NO: 23 - DNA, 336 bp, Artificial Sequence
  CD3z
cgcgtcaagttcagccgatcagccgatgctcctgcatacaagcagggccagaatcagctgtataacgagctgaatctggggcgccgagaggaatacgacgtgctggataagcggagagggagggaccccgaaatgggaggcaaacctaggcgcaagaacccacaggagggactgtacaatgaactgcagaaggacaaaatggccgaggcttattccgaaattgggatgaaaggagagcgacggagagggaagggacacgatgggctgtatcagggactgtctaccgccactaaagatacctacgacgctctgcacatgcaggctctgccacctcgc